European Patent Application EP 4 778 588 A2, published July 22, 2026. Title: ENZYMATICALLY CLEAVABLE LINKER AND LIGAND-ERIBULIN CONJUGATE CONTAINING SAME. Applicant: Innolake Biopharma (Hangzhou) Co., Ltd. Application CN PCZ/CN2023/121374, filed September 26, 2023. The sequence listing filed with the application follows.

SEQUENCE LISTING (19 sequences)

SEQ ID NO: 1 - protein, 5 aa, synthetic construct
SYAVS

SEQ ID NO: 2 - protein, 17 aa, synthetic construct
SISGGGIYIYYPDSVKG

SEQ ID NO: 3 - protein, 9 aa, synthetic construct
HGGAGYFDY

SEQ ID NO: 4 - protein, 11 aa, synthetic construct
RGSESVHSYLA

SEQ ID NO: 5 - protein, 7 aa, synthetic construct
NAKTLQS

SEQ ID NO: 6 - protein, 10 aa, synthetic construct
QQHYGSPPWT

SEQ ID NO: 7 - protein, 118 aa, synthetic construct
EVQLVESGGGLVKPGGSLRLSCAASGFTFSSYAVSWVRQAPGKGLEWVASISGGGIYIYYPDSVKGRFTISRDNAKNSLYLQMNSLRAEDTAVYYCARHGGAGYFDYWGQGTLVTVSS

SEQ ID NO: 8 - protein, 108 aa, synthetic construct
DSQMTQSPSSLSASVGDRVTITCRGSESVHSYLAWYQQKPGKAPKLLVYNAKTLQSGVPSRFSGSGSGTDFTLTISSLQPEDFATYYCQQHYGSPPWTFGGGTKVEIK

SEQ ID NO: 9 - protein, 330 aa, synthetic construct [sequence omitted]

SEQ ID NO: 10 - protein, 330 aa, synthetic construct
ASTKGPSVFPLAPSSKSTSGGTAALGCLVKDYFPEPVTVSWNSGALTSGVHTFPAVLQSSGLYSLSSVVTVPSSSLGTQTYICNVNHKPSNTKVDKKVEPKSCDKTHTSPPSPAPELLGGPSVFLFPPKPKDTLMISRTPEVTCVVVDVSHEDPEVKFNWYVDGVEVHNAKTKPREEQYNSTYRVVSVLTVLHQDWLNGKEYKCKVSNKALPAPIEKTISKAKGQPREPQVCTLPPCRDELTKNQVSLTCLVKGFYPSDIAVEWESNGQPENNYKTTPPVLDSDGSFFLYSKLTVDKSRWQQGNVFSCSVMHEALHNHYTQKSLSLSPGK

SEQ ID NO: 11 - protein, 107 aa, synthetic construct [sequence omitted]

SEQ ID NO: 12 - protein, 450 aa, synthetic construct
EVQLVESGGGLVQPGGSLRLSCAASGFNIKDTYIHWVRQAPGKGLEWVARIYPTNGYTRYADSVKGRFTISADTSKNTAYLQMNSLRAEDTAVYYCSRWGGDGFYAMDYWGQGTLVTVSSASTKGPSVFPLAPSSKSTSGGTAALGCLVKDYFPEPVTVSWNSGALTSGVHTFPAVLQSSGLYSLSSVVTVPSSSLGTQTYICNVNHKPSNTKVDKKVEPKSCDKTHTCPPCPAPELLGGPSVFLFPPKPKDTLMISRTPEVTCVVVDVSHEDPEVKFNWYVDGVEVHNAKTKPREEQYNSTYRVVSVLTVLHQDWLNGKEYKCKVSNKALPAPIEKTISKAKGQPREPQVYTLPPSREEMTKNQVSLTCLVKGFYPSDIAVEWESNGQPENNYKTTPPVLDSDGSFFLYSKLTVDKSRWQQGNVFSCSVMHEALHNHYTQKSLSLSPGK

SEQ ID NO: 13 - protein, 214 aa, synthetic construct
DIQMTQSPSSLSASVGDRVTITCRASQDVNTAVAWYQQKPGKAPKLLIYSASFLYSGVPSRFSGSRSGTDFTLTISSLQPEDFATYYCQQHYTTPPTFGQGTKVEIKRTVAAPSVFIFPPSDEQLKSGTASVVCLLNNFYPREAKVQWKVDNALQSGNSQESVTEQDSKDSTYSLSSTLTLSKADYEKHKVYACEVTHQGLSSPVTKSFNRGEC

SEQ ID NO: 14 - protein, 444 aa, synthetic construct
QVQLVQSGAEVKKPGSSVKVSCKASGYIFTTYNVHWVRQAPGQGLEWIGSIYPDNGDTSYNQNFKGRATITADKSTSTAYMELSSLRSEDTAVYYCARGDFAYWGQGTLVTVSSASTKGPSVFPLAPSSKSTSGGTAALGCLVKDYFPEPVTVSWNSGALTSGVHTFPAVLQSSGLYSLSSVVTVPSSSLGTQTYICNVNHKPSNTKVDKRVEPKSCDKTHTCPPCPAPELLGGPSVFLFPPKPKDTLMISRTPEVTCVVVDVSHEDPEVKFNWYVDGVEVHNAKTKPREEQYNSTYRVVSVLTVLHQDWLNGKEYKCKVSNKALPAPIEKTISKAKGQPREPQVYTLPPSREEMTKNQVSLTCLVKGFYPSDIAVEWESNGQPENNYKTTPPVLDSDGSFFLYSKLTVDKSRWQQGNVFSCSVMHEALHNHYTQKSLSLSPGK

SEQ ID NO: 15 - protein, 214 aa, synthetic construct
DIQMTQSPSSLSASVGDRVTITCKASQGVSNDVAWYQQKPGKAPKLLIYSASYRYTGVPSRFSGSGSGTDFTFTISSLQPEDIATYYCQQHSTTPYTFGQGTKLEIKRTVAAPSVFIFPPSDEQLKSGTASVVCLLNNFYPREAKVQWKVDNALQSGNSQESVTEQDSKDSTYSLSSTLTLSKADYEKHKVYACEVTHQGLSSPVTKSFNRGEC

SEQ ID NO: 16 - protein, 4 aa, synthetic construct
GGFG

SEQ ID NO: 17 - protein, 6 aa, synthetic construct
VAGGFG

SEQ ID NO: 18 - DNA, 72 bp, synthetic construct
  source 1..72: mol_type = other DNA
gaattcgccgccaccatgggatggtcctgtattatcctgttcctggtcgctaccgctaccggtgtccactca

SEQ ID NO: 19 - protein, 6 aa, synthetic construct
  VARIANT 1: note = G,A,V,L,I,P,F,Y,W,S,T,C,M,D,Q,N,K,R,E,H
  VARIANT 2: note = G,A,V,L,I,P,F,Y,W,S,T,C,M,D,Q,N,K,R, E, H
XXGGFG